European Patent Application EP 4 400 590 A1, published July 17, 2024. Title: Plasmid platform for stable expression and delivery of biomolecules. Applicant: kkoom lab. Application KR. The sequence listing filed with the application follows.

SEQUENCE LISTING (35 sequences)

SEQ ID NO: 1 - DNA, 1233 bp, synthetic construct
  misc_feature 1..1233: note = LAMP2
  source 1..1233: mol_type = other DNA
atggtgtgcttccgcctcttcccggttccgggctcagggctcgttctggtctgcctagtcctgggagctgtgcggtcttatgcattggaacttaatttgacagattcagaaaatgccacttgcctttatgcaaaatggcagatgaatttcacagttcgctatgaaactacaaataaaacttataaaactgtaaccatttcagaccatggcactgtgacatataatggaagcatttgtggggatgatcagaatggtcccaaaatagcagtgcagttcggacctggcttttcctggattgcgaattttaccaaggcagcatctacttattcaattgacagcgtctcattttcctacaacactggtgataacacaacatttcctgatgctgaagataaaggaattcttactgttgatgaacttttggccatcagaattccattgaatgacctttttagatgcaatagtttatcaactttggaaaagaatgatgttgtccaacactactgggatgttcttgtacaagcttttgtccaaaatggcacagtgagcacaaatgagttcctgtgtgataaagacaaaacttcaacagtggcacccaccatacacaccactgtgccatctcctactacaacacctactccaaaggaaaaaccagaagctggaacctattcagttaataatggcaatgatacttgcctgctggctaccatggggctgcagctgaacatcactcaggataaggttgcttcagttattaacatcaaccccaatacaactcactccacaggcagctgccgttctcacactgctctacttagactcaatagcagcactattaagtatctagactttgtctttgctgtgaaaaatgaaaaccgattttatctgaaggaagtgaacatcagcatgtatttggttaatggctccgttttcagcattgcaaataacaatctcagctactgggatgcccccctgggaagttcttatatgtgcaacaaagagcagactgtttcagtgtctggagcatttcagataaatacctttgatctaagggttcagcctttcaatgtgacacaaggaaagtattctacagcccaagagtgttcgctggatgatgacaccattctaatcccaattatagttggtgctggtctttcaggcttgattatcgttatagtgattgcttacgtaattggcagaagaaaaagttatgctggatatcagactctgtaa

SEQ ID NO: 2 - DNA, 1203 bp, synthetic construct
  misc_feature 1..1203: note = LAMP2-IC
  source 1..1203: mol_type = other DNA
atggtgtgcttccgcctcttcccggttccgggctcagggctcgttctggtctgcctagtcctgggagctgtgcggtcttatgcattggaacttaatttgacagattcagaaaatgccacttgcctttatgcaaaatggcagatgaatttcacagttcgctatgaaactacaaataaaacttataaaactgtaaccatttcagaccatggcactgtgacatataatggaagcatttgtggggatgatcagaatggtcccaaaatagcagtgcagttcggacctggcttttcctggattgcgaattttaccaaggcagcatctacttattcaattgacagcgtctcattttcctacaacactggtgataacacaacatttcctgatgctgaagataaaggaattcttactgttgatgaacttttggccatcagaattccattgaatgacctttttagatgcaatagtttatcaactttggaaaagaatgatgttgtccaacactactgggatgttcttgtacaagcttttgtccaaaatggcacagtgagcacaaatgagttcctgtgtgataaagacaaaacttcaacagtggcacccaccatacacaccactgtgccatctcctactacaacacctactccaaaggaaaaaccagaagctggaacctattcagttaataatggcaatgatacttgcctgctggctaccatggggctgcagctgaacatcactcaggataaggttgcttcagttattaacatcaaccccaatacaactcactccacaggcagctgccgttctcacactgctctacttagactcaatagcagcactattaagtatctagactttgtctttgctgtgaaaaatgaaaaccgattttatctgaaggaagtgaacatcagcatgtatttggttaatggctccgttttcagcattgcaaataacaatctcagctactgggatgcccccctgggaagttcttatatgtgcaacaaagagcagactgtttcagtgtctggagcatttcagataaatacctttgatctaagggttcagcctttcaatgtgacacaaggaaagtattctacagcccaagagtgttcgctggatgatgacaccattctaatcccaattatagttggtgctggtctttcaggcttgattatcgttatagtgattgcttacgtaattggcagataa

SEQ ID NO: 3 - DNA, 192 bp, synthetic construct
  misc_feature 1..192: note = LAMP2-EC
  source 1..192: mol_type = other DNA
atggtgtgcttccgcctcttcccggttccgggctcagggctcgttctggtctgcctagtcctgggagctgtgcggtcttatgcactaatcccaattatagttggtgctggtctttcaggcttgattatcgttatagtgattgcttacgtaattggcagaagaaaaagttatgctggatatcagactctgtaa

SEQ ID NO: 4 - DNA, 162 bp, synthetic construct
  misc_feature 1..162: note = LAMP2-EC/IC
  source 1..162: mol_type = other DNA
atggtgtgcttccgcctcttcccggttccgggctcagggctcgttctggtctgcctagtcctgggagctgtgcggtcttatgcactaatcccaattatagttggtgctggtctttcaggcttgattatcgttatagtgattgcttacgtaattggcagataa

SEQ ID NO: 5 - DNA, 2061 bp, synthetic construct
  misc_feature 1..2061: note = LAMP2-GFP
  source 1..2061: mol_type = other DNA
atggtgtgcttccgcctcttcccggttccgggctcagggctcgttctggtctgcctagtcctgggagctgtgcggtcttatgcagactataaagatgacgatgacaagggctcgagtttggaacttaatttgacagattcagaaaatgccacttgcctttatgcaaaatggcagatgaatttcacagttcgctatgaaactacaaataaaacttataaaactgtaaccatttcagaccatggcactgtgacatataatggaagcatttgtggggatgatcagaatggtcccaaaatagcagtgcagttcggacctggcttttcctggattgcgaattttaccaaggcagcatctacttattcaattgacagcgtctcattttcctacaacactggtgataacacaacatttcctgatgctgaagataaaggaattcttactgttgatgaacttttggccatcagaattccattgaatgacctttttagatgcaatagtttatcaactttggaaaagaatgatgttgtccaacactactgggatgttcttgtacaagcttttgtccaaaatggcacagtgagcacaaatgagttcctgtgtgataaagacaaaacttcaacagtggcacccaccatacacaccactgtgccatctcctactacaacacctactccaaaggaaaaaccagaagctggaacctattcagttaataatggcaatgatacttgcctgctggctaccatggggctgcagctgaacatcactcaggataaggttgcttcagttattaacatcaaccccaatacaactcactccacaggcagctgccgttctcacactgctctacttagactcaatagcagcactattaagtatctagactttgtctttgctgtgaaaaatgaaaaccgattttatctgaaggaagtgaacatcagcatgtatttggttaatggctccgttttcagcattgcaaataacaatctcagctactgggatgcccccctgggaagttcttatatgtgcaacaaagagcagactgtttcagtgtctggagcatttcagataaatacctttgatctaagggttcagcctttcaatgtgacacaaggaaagtattctacagcccaagagtgttcgctggatgatgacaccattctaatcccaattatagttggtgctggtctttcaggcttgattatcgttatagtgattgcttacgtaattggcagaagaaaaagttatgctggatatcagactctgggaagcggatacccatacgatgtgccagattacgctaagtcgacggtaccgcgggcccgggatccaccggtcgccaccatggtgagcaagggcgaggagctgttcaccggggtggtgcccatcctggtcgagctggacggcgacgtaaacggccacaagttcagcgtgtccggcgagggcgagggcgatgccacctacggcaagctgaccctgaagttcatctgcaccaccggcaagctgcccgtgccctggcccaccctcgtgaccaccctgacctacggcgtgcagtgcttcagccgctaccccgaccacatgaagcagcacgacttcttcaagtccgccatgcccgaaggctacgtccaggagcgcaccatcttcttcaaggacgacggcaactacaagacccgcgccgaggtgaagttcgagggcgacaccctggtgaaccgcatcgagctgaagggcatcgacttcaaggaggacggcaacatcctggggcacaagctggagtacaactacaacagccacaacgtctatatcatggccgacaagcagaagaacggcatcaaggtgaacttcaagatccgccacaacatcgaggacggcagcgtgcagctcgccgaccactaccagcagaacacccccatcggcgacggccccgtgctgctgcccgacaaccactacctgagcacccagtccgccctgagcaaagaccccaacgagaagcgcgatcacatggtcctgctggagttcgtgaccgccgccgggatcactctcggcatggacgagctgtacaagtaa

SEQ ID NO: 6 - DNA, 2040 bp, synthetic construct
  misc_feature 1..2040: note = LAMP2-IC-GFP
  source 1..2040: mol_type = other DNA
atggtgtgcttccgcctcttcccggttccgggctcagggctcgttctggtctgcctagtcctgggagctgtgcggtcttatgcagactataaagatgacgatgacaagggctcgagtttggaacttaatttgacagattcagaaaatgccacttgcctttatgcaaaatggcagatgaatttcacagttcgctatgaaactacaaataaaacttataaaactgtaaccatttcagaccatggcactgtgacatataatggaagcatttgtggggatgatcagaatggtcccaaaatagcagtgcagttcggacctggcttttcctggattgcgaattttaccaaggcagcatctacttattcaattgacagcgtctcattttcctacaacactggtgataacacaacatttcctgatgctgaagataaaggaattcttactgttgatgaacttttggccatcagaattccattgaatgacctttttagatgcaatagtttatcaactttggaaaagaatgatgttgtccaacactactgggatgttcttgtacaagcttttgtccaaaatggcacagtgagcacaaatgagttcctgtgtgataaagacaaaacttcaacagtggcacccaccatacacaccactgtgccatctcctactacaacacctactccaaaggaaaaaccagaagctggaacctattcagttaataatggcaatgatacttgcctgctggctaccatggggctgcagctgaacatcactcaggataaggttgcttcagttattaacatcaaccccaatacaactcactccacaggcagctgccgttctcacactgctctacttagactcaatagcagcactattaagtatctagactttgtctttgctgtgaaaaatgaaaaccgattttatctgaaggaagtgaacatcagcatgtatttggttaatggctccgttttcagcattgcaaataacaatctcagctactgggatgcccccctgggaagttcttatatgtgcaacaaagagcagactgtttcagtgtctggagcatttcagataaatacctttgatctaagggttcagcctttcaatgtgacacaaggaaagtattctacagcccaagagtgttcgctggatgatgacaccattctaatcccaattatagttggtgctggtctttcaggcttgattatcgttatagtgattgcttacgtaattggcagaggtagcggtggaagcggatacccatacgatgtgccagattacgctaagtcgacggtaccgcgggcccgggatccaccggtcgccaccatggtgagcaagggcgaggagctgttcaccggggtggtgcccatcctggtcgagctggacggcgacgtaaacggccacaagttcagcgtgtccggcgagggcgagggcgatgccacctacggcaagctgaccctgaagttcatctgcaccaccggcaagctgcccgtgccctggcccaccctcgtgaccaccctgacctacggcgtgcagtgcttcagccgctaccccgaccacatgaagcagcacgacttcttcaagtccgccatgcccgaaggctacgtccaggagcgcaccatcttcttcaaggacgacggcaactacaagacccgcgccgaggtgaagttcgagggcgacaccctggtgaaccgcatcgagctgaagggcatcgacttcaaggaggacggcaacatcctggggcacaagctggagtacaactacaacagccacaacgtctatatcatggccgacaagcagaagaacggcatcaaggtgaacttcaagatccgccacaacatcgaggacggcagcgtgcagctcgccgaccactaccagcagaacacccccatcggcgacggccccgtgctgctgcccgacaaccactacctgagcacccagtccgccctgagcaaagaccccaacgagaagcgcgatcacatggtcctgctggagttcgtgaccgccgccgggatcactctcggcatggacgagctgtacaagtaa

SEQ ID NO: 7 - DNA, 1035 bp, synthetic construct
  misc_feature 1..1035: note = LAMP2-EC-GFP
  source 1..1035: mol_type = other DNA
atggtgtgcttccgcctcttcccggttccgggctcagggctcgttctggtctgcctagtcctgggagctgtgcggtcttatgcagactataaagatgacgatgacaagggctcgagtggtggaggatctggtctaatcccaattatagttggtgctggtctttcaggcttgattatcgttatagtgattgcttacgtaattggcagaagaaaaagttatgctggatatcagactctgggaagcggatacccatacgatgtgccagattacgctaagtcgacggtaccgcgggcccgggatccaccggtcgccaccatggtgagcaagggcgaggagctgttcaccggggtggtgcccatcctggtcgagctggacggcgacgtaaacggccacaagttcagcgtgtccggcgagggcgagggcgatgccacctacggcaagctgaccctgaagttcatctgcaccaccggcaagctgcccgtgccctggcccaccctcgtgaccaccctgacctacggcgtgcagtgcttcagccgctaccccgaccacatgaagcagcacgacttcttcaagtccgccatgcccgaaggctacgtccaggagcgcaccatcttcttcaaggacgacggcaactacaagacccgcgccgaggtgaagttcgagggcgacaccctggtgaaccgcatcgagctgaagggcatcgacttcaaggaggacggcaacatcctggggcacaagctggagtacaactacaacagccacaacgtctatatcatggccgacaagcagaagaacggcatcaaggtgaacttcaagatccgccacaacatcgaggacggcagcgtgcagctcgccgaccactaccagcagaacacccccatcggcgacggccccgtgctgctgcccgacaaccactacctgagcacccagtccgccctgagcaaagaccccaacgagaagcgcgatcacatggtcctgctggagttcgtgaccgccgccgggatcactctcggcatggacgagctgtacaagtaa

SEQ ID NO: 8 - DNA, 1014 bp, synthetic construct
  misc_feature 1..1014: note = LAMP2-EC/IC-GFP
  source 1..1014: mol_type = other DNA
atggtgtgcttccgcctcttcccggttccgggctcagggctcgttctggtctgcctagtcctgggagctgtgcggtcttatgcagactataaagatgacgatgacaagggctcgagtggtggaggatctggtctaatcccaattatagttggtgctggtctttcaggcttgattatcgttatagtgattgcttacgtaattggcagaggtagcggtggaagcggatacccatacgatgtgccagattacgctaagtcgacggtaccgcgggcccgggatccaccggtcgccaccatggtgagcaagggcgaggagctgttcaccggggtggtgcccatcctggtcgagctggacggcgacgtaaacggccacaagttcagcgtgtccggcgagggcgagggcgatgccacctacggcaagctgaccctgaagttcatctgcaccaccggcaagctgcccgtgccctggcccaccctcgtgaccaccctgacctacggcgtgcagtgcttcagccgctaccccgaccacatgaagcagcacgacttcttcaagtccgccatgcccgaaggctacgtccaggagcgcaccatcttcttcaaggacgacggcaactacaagacccgcgccgaggtgaagttcgagggcgacaccctggtgaaccgcatcgagctgaagggcatcgacttcaaggaggacggcaacatcctggggcacaagctggagtacaactacaacagccacaacgtctatatcatggccgacaagcagaagaacggcatcaaggtgaacttcaagatccgccacaacatcgaggacggcagcgtgcagctcgccgaccactaccagcagaacacccccatcggcgacggccccgtgctgctgcccgacaaccactacctgagcacccagtccgccctgagcaaagaccccaacgagaagcgcgatcacatggtcctgctggagttcgtgaccgccgccgggatcactctcggcatggacgagctgtacaagtaa

SEQ ID NO: 9 - DNA, 516 bp, synthetic construct
  misc_feature 1..516: note = LEL-LAMP2-EC-GFP
  source 1..516: mol_type = other DNA
atggtgtgcttccgcctcttcccggttccgggctcagggctcgttctggtctgcctagtcctgggagctgtgcggtcttatgcagactataaagatgacgatgacaagggctcgagtggtggaggatctggttattcccacaaggatgaggtgattaaggaagtccaggagttttacaaggacacctacaacaagctgaaaaccaaggatgagccccagcgggaaacgctgaaagccatccactatgcgttgaactgctgtggtttggctgggggcgtggaacagtttatctcagacatctgccccaagaaggacgtactcgaaaccttcaccgtgaagtcctgtcctgatgccatcaaagaggtcttcgacctaatcccaattatagttggtgctggtctttcaggcttgattatcgttatagtgattgcttacgtaattggcagaagaaaaagttatgctggatatcagactctgggaagcggatacccatacgatgtgccagattacgcttaa

SEQ ID NO: 10 - DNA, 495 bp, synthetic construct
  misc_feature 1..495: note = LEL-LAMP2-EC/IC-GFP
  source 1..495: mol_type = other DNA
atggtgtgcttccgcctcttcccggttccgggctcagggctcgttctggtctgcctagtcctgggagctgtgcggtcttatgcagactataaagatgacgatgacaagggctcgagtggtggaggatctggttattcccacaaggatgaggtgattaaggaagtccaggagttttacaaggacacctacaacaagctgaaaaccaaggatgagccccagcgggaaacgctgaaagccatccactatgcgttgaactgctgtggtttggctgggggcgtggaacagtttatctcagacatctgccccaagaaggacgtactcgaaaccttcaccgtgaagtcctgtcctgatgccatcaaagaggtcttcgacctaatcccaattatagttggtgctggtctttcaggcttgattatcgttatagtgattgcttacgtaattggcagaggtagcggtggaagcggatacccatacgatgtgccagattacgcttaa

SEQ ID NO: 11 - DNA, 15 bp, synthetic construct
  misc_feature 1..15: note = GNSTM
  source 1..15: mol_type = other DNA
ggtaactcgactatg

SEQ ID NO: 12 - DNA, 69 bp, synthetic construct
  misc_feature 1..69: note = SEL
  source 1..69: mol_type = other DNA
ctccgattcgactctcagaccaagagcatcttcgagcaagaaactaataataataattccagcttctac

SEQ ID NO: 13 - skipped

SEQ ID NO: 14 - DNA, 2106 bp, synthetic construct
  misc_feature 1..2106: note = GNSTM-LAMP2-GFP
  source 1..2106: mol_type = other DNA
atggtgtgcttccgcctcttcccggttccgggctcagggctcgttctggtctgcctagtcctgggagctgtgcggtcttatgcaggtaactcgactatgggcagtggagactataaagatgacgatgacaagggcagtggatctggatccggtggctcgagtttggaacttaatttgacagattcagaaaatgccacttgcctttatgcaaaatggcagatgaatttcacagttcgctatgaaactacaaataaaacttataaaactgtaaccatttcagaccatggcactgtgacatataatggaagcatttgtggggatgatcagaatggtcccaaaatagcagtgcagttcggacctggcttttcctggattgcgaattttaccaaggcagcatctacttattcaattgacagcgtctcattttcctacaacactggtgataacacaacatttcctgatgctgaagataaaggaattcttactgttgatgaacttttggccatcagaattccattgaatgacctttttagatgcaatagtttatcaactttggaaaagaatgatgttgtccaacactactgggatgttcttgtacaagcttttgtccaaaatggcacagtgagcacaaatgagttcctgtgtgataaagacaaaacttcaacagtggcacccaccatacacaccactgtgccatctcctactacaacacctactccaaaggaaaaaccagaagctggaacctattcagttaataatggcaatgatacttgcctgctggctaccatggggctgcagctgaacatcactcaggataaggttgcttcagttattaacatcaaccccaatacaactcactccacaggcagctgccgttctcacactgctctacttagactcaatagcagcactattaagtatctagactttgtctttgctgtgaaaaatgaaaaccgattttatctgaaggaagtgaacatcagcatgtatttggttaatggctccgttttcagcattgcaaataacaatctcagctactgggatgcccccctgggaagttcttatatgtgcaacaaagagcagactgtttcagtgtctggagcatttcagataaatacctttgatctaagggttcagcctttcaatgtgacacaaggaaagtattctacagcccaagagtgttcgctggatgatgacaccattctaatcccaattatagttggtgctggtctttcaggcttgattatcgttatagtgattgcttacgtaattggcagaagaaaaagttatgctggatatcagactctgggaagcggatacccatacgatgtgccagattacgctaagtcgacggtaccgcgggcccgggatccaccggtcgccaccatggtgagcaagggcgaggagctgttcaccggggtggtgcccatcctggtcgagctggacggcgacgtaaacggccacaagttcagcgtgtccggcgagggcgagggcgatgccacctacggcaagctgaccctgaagttcatctgcaccaccggcaagctgcccgtgccctggcccaccctcgtgaccaccctgacctacggcgtgcagtgcttcagccgctaccccgaccacatgaagcagcacgacttcttcaagtccgccatgcccgaaggctacgtccaggagcgcaccatcttcttcaaggacgacggcaactacaagacccgcgccgaggtgaagttcgagggcgacaccctggtgaaccgcatcgagctgaagggcatcgacttcaaggaggacggcaacatcctggggcacaagctggagtacaactacaacagccacaacgtctatatcatggccgacaagcagaagaacggcatcaaggtgaacttcaagatccgccacaacatcgaggacggcagcgtgcagctcgccgaccactaccagcagaacacccccatcggcgacggccccgtgctgctgcccgacaaccactacctgagcacccagtccgccctgagcaaagaccccaacgagaagcgcgatcacatggtcctgctggagttcgtgaccgccgccgggatcactctcggcatggacgagctgtacaagtaa

SEQ ID NO: 15 - DNA, 2085 bp, synthetic construct
  misc_feature 1..2085: note = GNSTM-LAMP2-IC-GFP
  source 1..2085: mol_type = other DNA
atggtgtgcttccgcctcttcccggttccgggctcagggctcgttctggtctgcctagtcctgggagctgtgcggtcttatgcaggtaactcgactatgggcagtggagactataaagatgacgatgacaagggcagtggatctggatccggtggctcgagtttggaacttaatttgacagattcagaaaatgccacttgcctttatgcaaaatggcagatgaatttcacagttcgctatgaaactacaaataaaacttataaaactgtaaccatttcagaccatggcactgtgacatataatggaagcatttgtggggatgatcagaatggtcccaaaatagcagtgcagttcggacctggcttttcctggattgcgaattttaccaaggcagcatctacttattcaattgacagcgtctcattttcctacaacactggtgataacacaacatttcctgatgctgaagataaaggaattcttactgttgatgaacttttggccatcagaattccattgaatgacctttttagatgcaatagtttatcaactttggaaaagaatgatgttgtccaacactactgggatgttcttgtacaagcttttgtccaaaatggcacagtgagcacaaatgagttcctgtgtgataaagacaaaacttcaacagtggcacccaccatacacaccactgtgccatctcctactacaacacctactccaaaggaaaaaccagaagctggaacctattcagttaataatggcaatgatacttgcctgctggctaccatggggctgcagctgaacatcactcaggataaggttgcttcagttattaacatcaaccccaatacaactcactccacaggcagctgccgttctcacactgctctacttagactcaatagcagcactattaagtatctagactttgtctttgctgtgaaaaatgaaaaccgattttatctgaaggaagtgaacatcagcatgtatttggttaatggctccgttttcagcattgcaaataacaatctcagctactgggatgcccccctgggaagttcttatatgtgcaacaaagagcagactgtttcagtgtctggagcatttcagataaatacctttgatctaagggttcagcctttcaatgtgacacaaggaaagtattctacagcccaagagtgttcgctggatgatgacaccattctaatcccaattatagttggtgctggtctttcaggcttgattatcgttatagtgattgcttacgtaattggcagaggtagcggtggaagcggatacccatacgatgtgccagattacgctaagtcgacggtaccgcgggcccgggatccaccggtcgccaccatggtgagcaagggcgaggagctgttcaccggggtggtgcccatcctggtcgagctggacggcgacgtaaacggccacaagttcagcgtgtccggcgagggcgagggcgatgccacctacggcaagctgaccctgaagttcatctgcaccaccggcaagctgcccgtgccctggcccaccctcgtgaccaccctgacctacggcgtgcagtgcttcagccgctaccccgaccacatgaagcagcacgacttcttcaagtccgccatgcccgaaggctacgtccaggagcgcaccatcttcttcaaggacgacggcaactacaagacccgcgccgaggtgaagttcgagggcgacaccctggtgaaccgcatcgagctgaagggcatcgacttcaaggaggacggcaacatcctggggcacaagctggagtacaactacaacagccacaacgtctatatcatggccgacaagcagaagaacggcatcaaggtgaacttcaagatccgccacaacatcgaggacggcagcgtgcagctcgccgaccactaccagcagaacacccccatcggcgacggccccgtgctgctgcccgacaaccactacctgagcacccagtccgccctgagcaaagaccccaacgagaagcgcgatcacatggtcctgctggagttcgtgaccgccgccgggatcactctcggcatggacgagctgtacaagtaa

SEQ ID NO: 16 - DNA, 1044 bp, synthetic construct
  misc_feature 1..1044: note = GNSTM-LAMP2-EC/IC-GFP
  source 1..1044: mol_type = other DNA
atggtgtgcttccgcctcttcccggttccgggctcagggctcgttctggtctgcctagtcctgggagctgtgcggtcttatgcaggtaactcgactatgggcagtggagactataaagatgacgatgacaagggcagtggatctggatccggtggctcgagtctaatcccaattatagttggtgctggtctttcaggcttgattatcgttatagtgattgcttacgtaattggcagaggtagcggtggaagcggatacccatacgatgtgccagattacgctaagtcgacggtaccgcgggcccgggatccaccggtcgccaccatggtgagcaagggcgaggagctgttcaccggggtggtgcccatcctggtcgagctggacggcgacgtaaacggccacaagttcagcgtgtccggcgagggcgagggcgatgccacctacggcaagctgaccctgaagttcatctgcaccaccggcaagctgcccgtgccctggcccaccctcgtgaccaccctgacctacggcgtgcagtgcttcagccgctaccccgaccacatgaagcagcacgacttcttcaagtccgccatgcccgaaggctacgtccaggagcgcaccatcttcttcaaggacgacggcaactacaagacccgcgccgaggtgaagttcgagggcgacaccctggtgaaccgcatcgagctgaagggcatcgacttcaaggaggacggcaacatcctggggcacaagctggagtacaactacaacagccacaacgtctatatcatggccgacaagcagaagaacggcatcaaggtgaacttcaagatccgccacaacatcgaggacggcagcgtgcagctcgccgaccactaccagcagaacacccccatcggcgacggccccgtgctgctgcccgacaaccactacctgagcacccagtccgccctgagcaaagaccccaacgagaagcgcgatcacatggtcctgctggagttcgtgaccgccgccgggatcactctcggcatggacgagctgtacaagtaa

SEQ ID NO: 17 - DNA, 1113 bp, synthetic construct
  misc_feature 1..1113: note = SEL-LAMP2-EC-GFP
  source 1..1113: mol_type = other DNA
atggtgtgcttccgcctcttcccggttccgggctcagggctcgttctggtctgcctagtcctgggagctgtgcggtcttatgcagactataaagatgacgatgacaagggctcgagtggtggaggatctggtctccgattcgactctcagaccaagagcatcttcgagcaagaaactaataataataattccagcttctacacaggagtcctaatcccaattatagttggtgctggtctttcaggcttgattatcgttatagtgattgcttacgtaattggcagaagaaaaagttatgctggatatcagactctgggaagcggatacccatacgatgtgccagattacgctaagtcgacggtaccgcgggcccgggatccaccggtcgccaccatggtgagcaagggcgaggagctgttcaccggggtggtgcccatcctggtcgagctggacggcgacgtaaacggccacaagttcagcgtgtccggcgagggcgagggcgatgccacctacggcaagctgaccctgaagttcatctgcaccaccggcaagctgcccgtgccctggcccaccctcgtgaccaccctgacctacggcgtgcagtgcttcagccgctaccccgaccacatgaagcagcacgacttcttcaagtccgccatgcccgaaggctacgtccaggagcgcaccatcttcttcaaggacgacggcaactacaagacccgcgccgaggtgaagttcgagggcgacaccctggtgaaccgcatcgagctgaagggcatcgacttcaaggaggacggcaacatcctggggcacaagctggagtacaactacaacagccacaacgtctatatcatggccgacaagcagaagaacggcatcaaggtgaacttcaagatccgccacaacatcgaggacggcagcgtgcagctcgccgaccactaccagcagaacacccccatcggcgacggccccgtgctgctgcccgacaaccactacctgagcacccagtccgccctgagcaaagaccccaacgagaagcgcgatcacatggtcctgctggagttcgtgaccgccgccgggatcactctcggcatggacgagctgtacaagtaa

SEQ ID NO: 18 - DNA, 1092 bp, synthetic construct
  misc_feature 1..1092: note = SEL-LAMP2-EC/IC-GFP
  source 1..1092: mol_type = other DNA
atggtgtgcttccgcctcttcccggttccgggctcagggctcgttctggtctgcctagtcctgggagctgtgcggtcttatgcagactataaagatgacgatgacaagggctcgagtggtggaggatctggtctccgattcgactctcagaccaagagcatcttcgagcaagaaactaataataataattccagcttctacacaggagtcctaatcccaattatagttggtgctggtctttcaggcttgattatcgttatagtgattgcttacgtaattggcagaggtagcggtggaagcggatacccatacgatgtgccagattacgctaagtcgacggtaccgcgggcccgggatccaccggtcgccaccatggtgagcaagggcgaggagctgttcaccggggtggtgcccatcctggtcgagctggacggcgacgtaaacggccacaagttcagcgtgtccggcgagggcgagggcgatgccacctacggcaagctgaccctgaagttcatctgcaccaccggcaagctgcccgtgccctggcccaccctcgtgaccaccctgacctacggcgtgcagtgcttcagccgctaccccgaccacatgaagcagcacgacttcttcaagtccgccatgcccgaaggctacgtccaggagcgcaccatcttcttcaaggacgacggcaactacaagacccgcgccgaggtgaagttcgagggcgacaccctggtgaaccgcatcgagctgaagggcatcgacttcaaggaggacggcaacatcctggggcacaagctggagtacaactacaacagccacaacgtctatatcatggccgacaagcagaagaacggcatcaaggtgaacttcaagatccgccacaacatcgaggacggcagcgtgcagctcgccgaccactaccagcagaacacccccatcggcgacggccccgtgctgctgcccgacaaccactacctgagcacccagtccgccctgagcaaagaccccaacgagaagcgcgatcacatggtcctgctggagttcgtgaccgccgccgggatcactctcggcatggacgagctgtacaagtaa

SEQ ID NO: 19 - DNA, 1014 bp, synthetic construct
  misc_feature 1..1014: note = Gly-LAMP2-EC/IC-GFP
  source 1..1014: mol_type = other DNA
atggtgtgcttccgcctcttcccggttccgggctcagggctcgttctggtctgcctagtcctgggagctgtgcggtcttatgcagactataaagatgacgatgacaagggctcgagtggtaacggatctggtctaatcccaattatagttggtgctggtctttcaggcttgattatcgttatagtgattgcttacgtaattggcagaggtagcggtggaagcggatacccatacgatgtgccagattacgctaagtcgacggtaccgcgggcccgggatccaccggtcgccaccatggtgagcaagggcgaggagctgttcaccggggtggtgcccatcctggtcgagctggacggcgacgtaaacggccacaagttcagcgtgtccggcgagggcgagggcgatgccacctacggcaagctgaccctgaagttcatctgcaccaccggcaagctgcccgtgccctggcccaccctcgtgaccaccctgacctacggcgtgcagtgcttcagccgctaccccgaccacatgaagcagcacgacttcttcaagtccgccatgcccgaaggctacgtccaggagcgcaccatcttcttcaaggacgacggcaactacaagacccgcgccgaggtgaagttcgagggcgacaccctggtgaaccgcatcgagctgaagggcatcgacttcaaggaggacggcaacatcctggggcacaagctggagtacaactacaacagccacaacgtctatatcatggccgacaagcagaagaacggcatcaaggtgaacttcaagatccgccacaacatcgaggacggcagcgtgcagctcgccgaccactaccagcagaacacccccatcggcgacggccccgtgctgctgcccgacaaccactacctgagcacccagtccgccctgagcaaagaccccaacgagaagcgcgatcacatggtcctgctggagttcgtgaccgccgccgggatcactctcggcatggacgagctgtacaagtaa

SEQ ID NO: 20 - DNA, 1089 bp, synthetic construct
  misc_feature 1..1089: note = LAMP2-EC25IC-GFP
  source 1..1089: mol_type = other DNA
atggtgtgcttccgcctcttcccggttccgggctcagggctcgttctggtctgcctagtcctgggagctgtgcggtcttatgcagactataaagatgacgatgacaagggctcgagtggtggaggatctggtagggttcagcctttcaatgtgacacaaggaaagtattctacagcccaagagtgttcgctggatgatgacaccattctaatcccaattatagttggtgctggtctttcaggcttgattatcgttatagtgattgcttacgtaattggcagaggtagcggtggaagcggatacccatacgatgtgccagattacgctaagtcgacggtaccgcgggcccgggatccaccggtcgccaccatggtgagcaagggcgaggagctgttcaccggggtggtgcccatcctggtcgagctggacggcgacgtaaacggccacaagttcagcgtgtccggcgagggcgagggcgatgccacctacggcaagctgaccctgaagttcatctgcaccaccggcaagctgcccgtgccctggcccaccctcgtgaccaccctgacctacggcgtgcagtgcttcagccgctaccccgaccacatgaagcagcacgacttcttcaagtccgccatgcccgaaggctacgtccaggagcgcaccatcttcttcaaggacgacggcaactacaagacccgcgccgaggtgaagttcgagggcgacaccctggtgaaccgcatcgagctgaagggcatcgacttcaaggaggacggcaacatcctggggcacaagctggagtacaactacaacagccacaacgtctatatcatggccgacaagcagaagaacggcatcaaggtgaacttcaagatccgccacaacatcgaggacggcagcgtgcagctcgccgaccactaccagcagaacacccccatcggcgacggccccgtgctgctgcccgacaaccactacctgagcacccagtccgccctgagcaaagaccccaacgagaagcgcgatcacatggtcctgctggagttcgtgaccgccgccgggatcactctcggcatggacgagctgtacaagtaa

SEQ ID NO: 21 - DNA, 1119 bp, synthetic construct
  misc_feature 1..1119: note = GNSTM-LAMP2-EC25IC-GFP
  source 1..1119: mol_type = other DNA
atggtgtgcttccgcctcttcccggttccgggctcagggctcgttctggtctgcctagtcctgggagctgtgcggtcttatgcaggtaactcgactatgggcagtggagactataaagatgacgatgacaagggcagtggatctggatccggtggctcgagtagggttcagcctttcaatgtgacacaaggaaagtattctacagcccaagagtgttcgctggatgatgacaccattctaatcccaattatagttggtgctggtctttcaggcttgattatcgttatagtgattgcttacgtaattggcagaggtagcggtggaagcggatacccatacgatgtgccagattacgctaagtcgacggtaccgcgggcccgggatccaccggtcgccaccatggtgagcaagggcgaggagctgttcaccggggtggtgcccatcctggtcgagctggacggcgacgtaaacggccacaagttcagcgtgtccggcgagggcgagggcgatgccacctacggcaagctgaccctgaagttcatctgcaccaccggcaagctgcccgtgccctggcccaccctcgtgaccaccctgacctacggcgtgcagtgcttcagccgctaccccgaccacatgaagcagcacgacttcttcaagtccgccatgcccgaaggctacgtccaggagcgcaccatcttcttcaaggacgacggcaactacaagacccgcgccgaggtgaagttcgagggcgacaccctggtgaaccgcatcgagctgaagggcatcgacttcaaggaggacggcaacatcctggggcacaagctggagtacaactacaacagccacaacgtctatatcatggccgacaagcagaagaacggcatcaaggtgaacttcaagatccgccacaacatcgaggacggcagcgtgcagctcgccgaccactaccagcagaacacccccatcggcgacggccccgtgctgctgcccgacaaccactacctgagcacccagtccgccctgagcaaagaccccaacgagaagcgcgatcacatggtcctgctggagttcgtgaccgccgccgggatcactctcggcatggacgagctgtacaagtaa

SEQ ID NO: 22 - DNA, 1089 bp, synthetic construct
  misc_feature 1..1089: note = Gly-LAMP2-EC25IC-GFP
  source 1..1089: mol_type = other DNA
atggtgtgcttccgcctcttcccggttccgggctcagggctcgttctggtctgcctagtcctgggagctgtgcggtcttatgcagactataaagatgacgatgacaagggctcgagtggtaacggatctggtagggttcagcctttcaatgtgacacaaggaaagtattctacagcccaagagtgttcgctggatgatgacaccattctaatcccaattatagttggtgctggtctttcaggcttgattatcgttatagtgattgcttacgtaattggcagaggtagcggtggaagcggatacccatacgatgtgccagattacgctaagtcgacggtaccgcgggcccgggatccaccggtcgccaccatggtgagcaagggcgaggagctgttcaccggggtggtgcccatcctggtcgagctggacggcgacgtaaacggccacaagttcagcgtgtccggcgagggcgagggcgatgccacctacggcaagctgaccctgaagttcatctgcaccaccggcaagctgcccgtgccctggcccaccctcgtgaccaccctgacctacggcgtgcagtgcttcagccgctaccccgaccacatgaagcagcacgacttcttcaagtccgccatgcccgaaggctacgtccaggagcgcaccatcttcttcaaggacgacggcaactacaagacccgcgccgaggtgaagttcgagggcgacaccctggtgaaccgcatcgagctgaagggcatcgacttcaaggaggacggcaacatcctggggcacaagctggagtacaactacaacagccacaacgtctatatcatggccgacaagcagaagaacggcatcaaggtgaacttcaagatccgccacaacatcgaggacggcagcgtgcagctcgccgaccactaccagcagaacacccccatcggcgacggccccgtgctgctgcccgacaaccactacctgagcacccagtccgccctgagcaaagaccccaacgagaagcgcgatcacatggtcctgctggagttcgtgaccgccgccgggatcactctcggcatggacgagctgtacaagtaa

SEQ ID NO: 23 - DNA, 637 bp, synthetic construct
  misc_feature 1..637: note = GNSTM-LAMP2-EC/IC-shGFP
  source 1..637: mol_type = other DNA
atggtgtgcttccgcctcttcccggttccgggctcagggctcgttctggtctgcctagtcctgggagctgtgcggtcttatgcaggtaactcgactatgggcagtggagactataaagatgacgatgacaagggcagtggatctggatccggtggctcgagtctaatcccaattatagttggtgctggtctttcaggcttgattatcgttatagtgattgcttacgtaattggcagaggtagcggtggaagcggatacccatacgatgtgccagattacgctggatcgggtaggcaccaggtaggggagctggctgggtggggcagccccgggaaggggggaaagctgaatgcaacccctggtgcaggaagggaggcttttcctgaggaccgggagaggattttaagtacatagaaggaagcttctggagatcctgctccgtcgccgtctatatcatggccgacatctctgagcctgggagctctgtcggccatgatatagacgttagactgggcaagggagagcaacgccatggaccgctggggacaaaatgggctgtttccaaggagaagacatttgtttgctccttttttgattcttgtcctttccttcccagggcgtgatgggcagcggctaa

SEQ ID NO: 24 - DNA, 688 bp, synthetic construct
  misc_feature 1..688: note = GNSTM-LAMP2-EC/IC-shGFP-BIV
  source 1..688: mol_type = other DNA
atggtgtgcttccgcctcttcccggttccgggctcagggctcgttctggtctgcctagtcctgggagctgtgcggtcttatgcaggtaactcgactatgggcagtggagactataaagatgacgatgacaagggcagtggatctggatccggtggctcgagtctaatcccaattatagttggtgctggtctttcaggcttgattatcgttatagtgattgcttacgtaattggcagaggtagcggtggaagcggatacccatacgatgtgccagattacgctggatcgggtaggcaccaggtaggggagctggctgggtggggcagccccgggaaggggggaaagctgaatgcaacccctggtgcaggaagggaggcttttcctgaggaccgggagaggattttaagtacatagaaggaagcttctggagatcctgctccgtcgccgtctatatcatggccgacatctctgagcctgggagctctgtcggccatgatatagacgttagactgggcaagggagagcaacgccatggaccgctggggacaaaatgggctgtttccaaggagaagacatttgtttgctccttttttgattcttgtcctttccttcccagggcgtgatgggcagcggcggcagcggccgaccacgtgggacacgcggcaagggccggcgcattaggcggtaa

SEQ ID NO: 25 - DNA, 700 bp, synthetic construct
  misc_feature 1..700: note = GNSTM-LAMP2-EC/IC-shGFP-JDV(WT)
  source 1..700: mol_type = other DNA
atggtgtgcttccgcctcttcccggttccgggctcagggctcgttctggtctgcctagtcctgggagctgtgcggtcttatgcaggtaactcgactatgggcagtggagactataaagatgacgatgacaagggcagtggatctggatccggtggctcgagtctaatcccaattatagttggtgctggtctttcaggcttgattatcgttatagtgattgcttacgtaattggcagaggtagcggtggaagcggatacccatacgatgtgccagattacgctggatcgggtaggcaccaggtaggggagctggctgggtggggcagccccgggaaggggggaaagctgaatgcaacccctggtgcaggaagggaggcttttcctgaggaccgggagaggattttaagtacatagaaggaagcttctggagatcctgctccgtcgccgtctatatcatggccgacatctctgagcctgggagctctgtcggccatgatatagacgttagactgggcaagggagagcaacgccatggaccgctggggacaaaatgggctgtttccaaggagaagacatttgtttgctccttttttgattcttgtcctttccttcccagggcgtgatgggcagcggcggcagcggccgacgaaaaaagcgtgggacacgcggcaagggccggaagattcactattaacggtaa

SEQ ID NO: 26 - DNA, 694 bp, synthetic construct
  misc_feature 1..694: note = GNSTM-LAMP2-EC/IC-shGFP-JDV(MT)
  source 1..694: mol_type = other DNA
atggtgtgcttccgcctcttcccggttccgggctcagggctcgttctggtctgcctagtcctgggagctgtgcggtcttatgcaggtaactcgactatgggcagtggagactataaagatgacgatgacaagggcagtggatctggatccggtggctcgagtctaatcccaattatagttggtgctggtctttcaggcttgattatcgttatagtgattgcttacgtaattggcagaggtagcggtggaagcggatacccatacgatgtgccagattacgctggatcgggtaggcaccaggtaggggagctggctgggtggggcagccccgggaaggggggaaagctgaatgcaacccctggtgcaggaagggaggcttttcctgaggaccgggagaggattttaagtacatagaaggaagcttctggagatcctgctccgtcgccgtctatatcatggccgacatctctgagcctgggagctctgtcggccatgatatagacgttagactgggcaagggagagcaacgccatggaccgctggggacaaaatgggctgtttccaaggagaagacatttgtttgctccttttttgattcttgtcctttccttcccagggcgtgatgggcagcggcggcagcggccgacgaaaaaagcgtgggacacgcggcaagggccggcgcattaggcggtaa

SEQ ID NO: 27 - DNA, 393 bp, synthetic construct
  misc_feature 1..393: note = SEL-LAMP2-EC/IC-BIV
  source 1..393: mol_type = other DNA
atggtgtgcttccgcctcttcccggttccgggctcagggctcgttctggtctgcctagtcctgggagctgtgcggtcttatgcagactataaagatgacgatgacaagggctcgagtggtggaggatctggtctccgattcgactctcagaccaagagcatcttcgagcaagaaactaataataataattccagcttctacacaggagtcctaatcccaattatagttggtgctggtctttcaggcttgattatcgttatagtgattgcttacgtaattggcagaggtagcggtggaagcggatacccatacgatgtgccagattacgctggcagcggcggcagcggccgaccacgtgggacacgcggcaagggccggcgcattaggcggtaa

SEQ ID NO: 28 - DNA, 736 bp, synthetic construct
  misc_feature 1..736: note = SEL-LAMP2-EC/IC-(Pri-miRNA-199)-BIV
  source 1..736: mol_type = other DNA
atggtgtgcttccgcctcttcccggttccgggctcagggctcgttctggtctgcctagtcctgggagctgtgcggtcttatgcagactataaagatgacgatgacaagggctcgagtggtggaggatctggtctccgattcgactctcagaccaagagcatcttcgagcaagaaactaataataataattccagcttctacacaggagtcctaatcccaattatagttggtgctggtctttcaggcttgattatcgttatagtgattgcttacgtaattggcagaggtagcggtggaagcggatacccatacgatgtgccagattacgctggatcgggtaggcaccaggtaggggagctggctgggtggggcagccccgggaaggggggaaagctgaatgcaacccctggtgcaggaagggaggcttttcctgaggaccgggagaggattttaagtacatagaaggaagcttctggagatcctgctccgtcgccccagtgttcagactacctgttctctgagcctgggagctcacagtagtctgcacattggttagactgggcaagggagagcaacgccatggaccgctggggacaaaatgggctgtttccaaggagaagacatttgtttgctccttttttgattcttgtcctttccttcccagggcgtgatgggcagcggcggcagcggccgaccacgtgggacacgcggcaagggccggcgcattaggcggtaa

SEQ ID NO: 29 - DNA, 637 bp, synthetic construct
  misc_feature 1..637: note = GNSTM-LAMP2-EC/IC-scramble shGFP
  source 1..637: mol_type = other DNA
atggtgtgcttccgcctcttcccggttccgggctcagggctcgttctggtctgcctagtcctgggagctgtgcggtcttatgcaggtaactcgactatgggcagtggagactataaagatgacgatgacaagggcagtggatctggatccggtggctcgagtctaatcccaattatagttggtgctggtctttcaggcttgattatcgttatagtgattgcttacgtaattggcagaggtagcggtggaagcggatacccatacgatgtgccagattacgctggatcgggtaggcaccaggtaggggagctggctgggtggggcagccccgggaaggggggaaagctgaatgcaacccctggtgcaggaagggaggcttttcctgaggaccgggagaggattttaagtacatagaaggaagcttctggagatcctgctccgtcgcctaaggttaagtcgccctcgtctctgagcctgggagctccgagggcgacttaaccttagttagactgggcaagggagagcaacgccatggaccgctggggacaaaatgggctgtttccaaggagaagacatttgtttgctccttttttgattcttgtcctttccttcccagggcgtgatgggcagcggctaa

SEQ ID NO: 30 - DNA, 210 bp, synthetic construct
  misc_feature 1..210: note = Double stranded RNA Binding Domain motif(DRBD)
  source 1..210: mol_type = other DNA
ttcttcatggaggaacttaatacataccgtcagaagcagggagtagtacttaaatatcaagaactgcctaattcaggacctccacatgataggaggtttacatttcaagttataatagatggaagagaatttccagaaggtgaaggtagatcaaagaaggaagcaaaaaatgccgcagccaaattagctgttgagatacttaataaggaa

SEQ ID NO: 31 - DNA, 42 bp, synthetic construct
  misc_feature 1..42: note = BIV derived RBD
  source 1..42: mol_type = other DNA
cgaccacgtgggacacgcggcaagggccggcgcattaggcgg

SEQ ID NO: 32 - DNA, 51 bp, synthetic construct
  misc_feature 1..51: note = JDV derived RBD
  source 1..51: mol_type = other DNA
cgacgaaaaaagcgtgggacacgcggcaagggccggaagattcactattaa

SEQ ID NO: 33 - DNA, 48 bp, synthetic construct
  misc_feature 1..48: note = JDV derived mutation RBD
  source 1..48: mol_type = other DNA
cgacgaaaaaagcgtgggacacgcggcaagggccggcgcattaggcgg

SEQ ID NO: 34 - DNA, 27 bp, synthetic construct
  misc_feature 1..27: note = HIV derived RBD
  source 1..27: mol_type = other DNA
aggaagaagaggaggcagaggaggagg

SEQ ID NO: 35 - DNA, 1056 bp, synthetic construct
  misc_feature 1..1056: note = GNSTM-LAMP2-EC/IC-SKOV3
  source 1..1056: mol_type = other DNA
atggtgtgcttccgcctcttcccggttccgggctcagggctcgttctggtctgcctagtcctgggagctgtgcggtcttatgcaggtaactcgactatgggcagtggaatgcataccgcaccgggatggggctataacctgtcgggcagtggatctggatccggtggctcgagtctaatcccaattatagttggtgctggtctttcaggcttgattatcgttatagtgattgcttacgtaattggcagaggtagcggtggaagcggatacccatacgatgtgccagattacgctaagtcgacggtaccgcgggcccgggatccaccggtcgccaccatggtgagcaagggcgaggagctgttcaccggggtggtgcccatcctggtcgagctggacggcgacgtaaacggccacaagttcagcgtgtccggcgagggcgagggcgatgccacctacggcaagctgaccctgaagttcatctgcaccaccggcaagctgcccgtgccctggcccaccctcgtgaccaccctgacctacggcgtgcagtgcttcagccgctaccccgaccacatgaagcagcacgacttcttcaagtccgccatgcccgaaggctacgtccaggagcgcaccatcttcttcaaggacgacggcaactacaagacccgcgccgaggtgaagttcgagggcgacaccctggtgaaccgcatcgagctgaagggcatcgacttcaaggaggacggcaacatcctggggcacaagctggagtacaactacaacagccacaacgtctatatcatggccgacaagcagaagaacggcatcaaggtgaacttcaagatccgccacaacatcgaggacggcagcgtgcagctcgccgaccactaccagcagaacacccccatcggcgacggccccgtgctgctgcccgacaaccactacctgagcacccagtccgccctgagcaaagaccccaacgagaagcgcgatcacatggtcctgctggagttcgtgaccgccgccgggatcactctcggcatggacgagctgtacaagtaa